European Patent Specification EP 3 575 318 B1, published September 4, 2024. Title: Anti-PD-1 Antibody and Use Thereof. Applicant: AMPSOURCE BIOPHARMA SHANGHAI INC. The sequence listing filed with the application follows.

SEQUENCE LISTING (42 sequences)

SEQ ID NO: 1 - protein, 8 aa, Artificial Sequence
  CDR-H1
GFTFSSYG

SEQ ID NO: 2 - protein, 8 aa, Artificial Sequence
  CDR-H1
GITFSNSG

SEQ ID NO: 3 - protein, 8 aa, Artificial Sequence
  CDR-H2
ISGGGRDT

SEQ ID NO: 4 - protein, 7 aa, Artificial Sequence
  CDR-H2
WYDGSKR

SEQ ID NO: 5 - protein, 11 aa, Artificial Sequence
  CDR-H3
ARQKDTSWFVH

SEQ ID NO: 6 - protein, 6 aa, Artificial Sequence
  CDR-H3
ATNDDY

SEQ ID NO: 7 - protein, 10 aa, Artificial Sequence
  CDR-L1
ESVDDYGISF

SEQ ID NO: 8 - protein, 6 aa, Artificial Sequence
  CDR-L1
QSVSSY

SEQ ID NO: 9 - protein, 3 aa, Artificial Sequence
  mAb1 CDR-L2
VAS

SEQ ID NO: 10 - protein, 3 aa, Artificial Sequence
  CDR-L2
DAS

SEQ ID NO: 11 - protein, 9 aa, Artificial Sequence
  CDR-L3
QQSKEVPWT

SEQ ID NO: 12 - protein, 9 aa, Artificial Sequence
  CDR-L3
QQSSNWPRT

SEQ ID NO: 13 - protein, 118 aa, Artificial Sequence
  Amino acid sequence of the heavy chain variable region of the murine antibody AB12M1 or the chimeric antibody AB12M2
EVKLVESGGGLVKPGGSLKLSCAASGFTFSSYGMSWVRQTPEKRLEWVATISGGGRDTYYPDSVKGRFTISRDNAKNNLYLQMSSLRSEDTALYYCARQKDTSWFVHWGQGTLVTVSA

SEQ ID NO: 14 - protein, 111 aa, Artificial Sequence
  Amino acid sequence of the light chain variable region of the murine antibody AB12M1 or the chimeric antibody AB12M2
DIVLTQSPASLAVSLGQRATISCRASESVDDYGISFMNWFQQKPGQPPKLLIYVASNQGSGVPARFSGSGSGTDFSLNIHPMEEDDTAMYFCQQSKEVPWTFGGGTKLEIK

SEQ ID NO: 15 - protein, 111 aa, Artificial Sequence
  Amino acid sequence of the heavy chain variable region of the murine antibody AB12N1 or the chimeric antibody AB12N2
QVQLVESGGGVVQPGRSLRLDCKASGITFSNSGMHWVRQAPGKGLEWVAVIWYDGSKRYYADSVKGRFTISRDNSKNTLFLQMNSLRAEDTAVYYCATNDDYWGQGTLVTV

SEQ ID NO: 16 - protein, 107 aa, Artificial Sequence [sequence omitted]

SEQ ID NO: 17 - protein, 118 aa, Artificial Sequence
  Amino acid sequence of the heavy chain variable region of humanized antibody AB12M3
EVQLVESGGGLVQPGGSLRLSCAASGFTFSSYGMSWVRQAPGKGLEWVATISGGGRDTYYPDSVKGRFTISRDNAKNNLYLQMNSLRAEDTALYYCARQKDTSWFVHWGQGTLVTVSS

SEQ ID NO: 18 - protein, 111 aa, Artificial Sequence
  Amino acid sequence of the light chain variable region of humanized antibody AB12M3
EIVLTQSPATLSLSPGERATLSCRASESVDDYGISFMNWFQQKPGQAPKLLIYVASNQGSGVPARFSGSGSGTDFSLTISSLEPDDTAMYFCQQSKEVPWTFGGGTKVEIK

SEQ ID NO: 19 - protein, 118 aa, Artificial Sequence
  Amino acid sequence of the heavy chain variable region of humanized antibody AB12M4
EVKLVESGGGLVKPGGSLRLSCAASGFTFSSYGMSWVRQTPEKRLEWVATISGGGRDTYYPDSVKGRFTISRDNAKNNLYLQMSSLRSEDTALYYCARQKDTSWFVHWGQGTLVTVSA

SEQ ID NO: 20 - protein, 111 aa, Artificial Sequence
  Amino acid sequence of the light chain variable region of humanized antibody AB12M4
EIVLTQSPATLAVSPGERATISCRASESVDDYGISFMNWFQQKPGQPPKLLIYVASNQGSGVPARFSGSGSGTDFTLNIHPMEEDDTAMYFCQQSKEVPWTFGGGTKLEIK

SEQ ID NO: 21 - protein, 118 aa, Artificial Sequence
  Amino acid sequence of the heavy chain variable region of humanized antibody AB12M5
EVQLVESGGGLVQPGGSLRLSCAASGFTFSSYGMSWVRQAPGKGLEWVSAISGGGRDTYYADSVKGRFTISRDNSKNTLYLQMNSLRAEDTAVYYCARQKDTSWFVHWGQGTMVTVSS

SEQ ID NO: 22 - protein, 107 aa, Artificial Sequence
  Amino acid sequence of the light chain variable region of humanized antibody AB12M5
EIVLTQSPATLSLSPGERATLSCRASESVDDYGISFLAWYQQKPGQAPRVASNRATGIPARFSGSGPGTDFTLTISSLEPEDFAVYYCQQSKEVPWTFGGGTKVEIK

SEQ ID NO: 23 - protein, 118 aa, Artificial Sequence
  Amino acid sequence of the heavy chain variable region of humanized antibody AB12M6
EVQLVESGGGLVQPGGSLRLSCAASGFTFSSYGMSWVRQAPEKGLEWVSAISGGGRDTYYADSVKGRFTISRDNSKNTLYLQMNSLRAEDTAVYYCARQKDTSWFVHWGQGTMVTVSS

SEQ ID NO: 24 - protein, 107 aa, Artificial Sequence
  Amino acid sequence of the light chain variable region of humanized antibody AB12M6
EIVLTQSPATLSLSPGERATLSCRASESVDDYGISFLAWFQQKPGQAPRVASNRASGIPARFSGSGPGTDFTLTISSLEPEDFAVYYCQQSKEVPWTFGGGTKVEIK

SEQ ID NO: 25 - protein, 118 aa, Artificial Sequence; identical to SEQ ID NO: 23
  Amino acid sequence of the heavy chain variable region of humanized antibody AB12M7

SEQ ID NO: 26 - protein, 107 aa, Artificial Sequence
  Amino acid sequence of the light chain variable region of humanized antibody AB12M7
DIVLTQSPATLSLSPGERATLSCRASESVDDYGISFLAWFQQKPGQAPRVASNRASGIPARFSGSGPGTDFTLTISSLEPDDFAVYYCQQSKEVPWTFGGGTKVEIK

SEQ ID NO: 27 - protein, 118 aa, Artificial Sequence; identical to SEQ ID NO: 23
  Amino acid sequence of the heavy chain variable region of humanized antibody AB12M8

SEQ ID NO: 28 - protein, 107 aa, Artificial Sequence
  Amino acid sequence of the light chain variable region of humanized antibody AB12M8
DIVLTQSPATLSLSPGERATLSCRASESVDDYGISFLAWYQQKPGQAPRVASNRASGIPARFSGSGSGTDFTLTISSLEPDDFAVYYCQQSKEVPWTFGGGTKVEIK

SEQ ID NO: 29 - protein, 118 aa, Artificial Sequence
  Amino acid sequence of the heavy chain variable region of humanized antibody AB12M9
EVKLVESGGGLVQPGGSLRLSCAASGFTFSSYGMSWVRQAPEKGLEWVSAISGGGRDTYYADSVKGRFTISRDNSKNTLYLQMNSLRAEDTALYYCARQKDTSWFVHWGQGTMVTVSS

SEQ ID NO: 30 - protein, 107 aa, Artificial Sequence; identical to SEQ ID NO: 28
  Amino acid sequence of the light chain variable region of humanized antibody AB12M9

SEQ ID NO: 31 - protein, 110 aa, Artificial Sequence
  Amino acid sequence of the heavy chain variable region of humanized antibody AB12N3
QVQLVESGGGVVQPGRSLRLSCAASGITFSNSGMHWVRQAPGKGLEWVAVWYDGSKRYYADSVKGRFTISRDNSKNTLYLQMNSLRAEDTAVYYCATNDDYWGQGTLVTV

SEQ ID NO: 32 - protein, 107 aa, Artificial Sequence [sequence omitted]

SEQ ID NO: 33 - protein, 111 aa, Artificial Sequence
  Amino acid sequence of the heavy chain variable region of humanized antibody AB12N4
QVQLVESGGGVVQPGRSLRLSCAASGITFSNSGMHWVRQAPGKGLEWVAVIWYDGSKRYYADSVKGRFTISRDNSKNTLYLQMNSLRAEDTAVYYCATNDDYWGQGTLVTV

SEQ ID NO: 34 - protein, 107 aa, Artificial Sequence [sequence omitted]

SEQ ID NO: 35 - protein, 110 aa, Artificial Sequence
  Amino acid sequence of the heavy chain variable region of humanized antibody AB12N5
QVQLVESGGGVVQPGRSLRLSCAASGITFSNSGMHWVRQAPGKGLEWVAVWYDGSKRYYADSVKGRFTISRDNSKNTLFLQMNSLRAEDTAVYYCATNDDYWGQGTLVTV

SEQ ID NO: 36 - protein, 107 aa, Artificial Sequence [sequence omitted]

SEQ ID NO: 37 - DNA, 354 bp, Artificial Sequence
  Nucleotide sequence of the heavy chain variable region of the chimeric antibody AB12M2
gaggtgaagctggtggagagcggaggaggactggtgaagccaggaggatctctgaagctgagctgtgctgcctctggcttcaccttttcctcttacggcatgagctgggtgagacagacacccgagaagcgcctggaatgggtcgctaccatctctggcggcggcagagacacatactatcctgattccgtgaagggcagattcaccatcagccgcgataacgccaaaaataatctgtatctgcaaatgtcttccctgaggtctgaggacaccgctctgtactattgcgcccggcagaaggatacatcttggttcgtgcactggggacagggcaccctggtgaccgtgtccgcc

SEQ ID NO: 38 - DNA, 333 bp, Artificial Sequence
  Nucleotide sequence of the light chain variable region of the chimeric antibody AB12M2
gacatcgtgctgacccagtctccagctagcctggccgtgtccctgggacagagggctaccatcagctgtcgggcctctgagtctgtcgacgattacggcatctctttcatgaattggttccagcagaaacctggccagccccctaaactgctgatctatgtcgcttccaatcagggaagcggagtgcctgctagattcagcggatctggatctggaaccgacttcagcctgaacatccatccaatggaggaggacgataccgccatgtacttctgtcagcagtctaaagaagtcccttggacctttggcggcggcacaaagctggagatcaag

SEQ ID NO: 39 - DNA, 354 bp, Artificial Sequence
  Nucleotide sequence of the heavy chain variable region of humanized antibody AB12M3
gaggtgcagctggtggagtccggaggaggactggtgcagcctggaggcagcctgagactgtcttgcgccgcttccggcttcaccttttccagctacggcatgtcttgggtgagacaggctcctggcaagggactggagtgggtggctaccatctccggaggaggaagggacacatactatccagatagcgtgaagggcaggttcacaatctctcgggacaacgctaagaacaatctgtatctgcagatgaactccctgagagctgaggacaccgccctgtactattgcgcccgccagaaggatacaagctggtttgtgcactggggccagggcaccctggtgacagtgtcttcc

SEQ ID NO: 40 - DNA, 333 bp, Artificial Sequence
  Nucleotide sequence of the light chain variable region of humanized antibody AB12M3
gagatcgtgctgacccagagccctgccacactgagcctgtctccaggcgagagggctaccctgtcttgtcgggcctccgagagcgtggacgattacggcatctccttcatgaactggtttcagcagaagccaggccaggctcccaagctgctgatctatgtggccagcaatcagggctctggagtgccagctcgcttctctggctccggaagcggaaccgacttttctctgacaatcagctctctggagccagacgatacagccatgtacttctgccagcagtccaaggaggtgccatggacctttggcggaggaacaaaggtggagatcaag

SEQ ID NO: 41 - DNA, 354 bp, Artificial Sequence
  Nucleotide sequence of the heavy chain variable region of humanized antibody AB12M4
gaggtgcagctggtggagagcggaggaggactggtgaagccaggaggatctctgaggctgagctgtgctgcctctggcttcaccttttcctcttacggcatgagctgggtgagacagacacccgagaagcgcctggaatgggtcgctaccatctctggcggcggcagagacacatactatcctgattccgtgaagggcagattcaccatcagccgcgataacgccaaaaataatctgtatctgcaaatgtcttccctgaggtctgaggacaccgctctgtactattgcgcccggcagaaggatacatcttggttcgtgcactggggacagggcaccctggtgaccgtgtcctcc

SEQ ID NO: 42 - DNA, 333 bp, Artificial Sequence
  Nucleotide sequence of the light chain variable region of humanized antibody AB12M4
gaaatcgtgctgacccagtctccagctacactggccgtgtcccctggagagagggctaccatcagctgtcgggcctctgagtctgtcgacgattacggcatctctttcatgaattggttccagcagaaacctggccagccccctaaactgctgatctatgtcgcttccaatcagggaagcggagtgcctgctagattcagcggatctggatctggaaccgacttcaccctgaacatccatccaatggaggaggacgataccgccatgtacttctgtcagcagtctaaagaagtcccttggacctttggcggcggcacaaagctggagatcaag